European Patent Application EP 4 278 891 A1, published November 22, 2023. Title: CLUBROOT RESISTANCE AND MARKERS IN BRASSICA. Applicant: KWS SAAT SE & Co. KGaA. The sequence listing filed with the application follows.

SEQUENCE LISTING (293 sequences)

SEQ ID NO: 1 - DNA, 42 bp, Artificial Sequence
  ra36387s01, primer allele X
gaaggtgaccaagttcatgctcggagacgaatttggagtggc

SEQ ID NO: 2 - DNA, 50 bp, Artificial Sequence
  ra36444s01, primer allele X
gaaggtgaccaagttcatgctcaatgcttcaagtaacacatttagaaacg

SEQ ID NO: 3 - DNA, 54 bp, Artificial Sequence
  ra36450s01, primer allele X
gaaggtgaccaagttcatgctatattayaatgactatgaattttgctaaccata

SEQ ID NO: 4 - DNA, 42 bp, Artificial Sequence
  ra36451s01, primer allele X
gaaggtgaccaagttcatgcttctgcgggaggagagcttctt

SEQ ID NO: 5 - DNA, 51 bp, Artificial Sequence
  ra36458s01, primer allele X
gaaggtgaccaagttcatgctattgattgarttcattctgttttcggttta

SEQ ID NO: 6 - DNA, 45 bp, Artificial Sequence
  ra36459s01, primer allele X
gaaggtgaccaagttcatgctgggtggttacaagataaggtacca

SEQ ID NO: 7 - DNA, 49 bp, Artificial Sequence
  ra36460s01, primer allele X
gaaggtgaccaagttcatgctgaacaaagatttccacgccaaaattcta

SEQ ID NO: 8 - DNA, 48 bp, Artificial Sequence
  ra36461s01, primer allele X
gaaggtgaccaagttcatgctcatcggacactctacatctttaagtta

SEQ ID NO: 9 - DNA, 48 bp, Artificial Sequence
  ra36463s01, primer allele X
gaaggtgaccaagttcatgctataggaacttatgaatctaacgttccg

SEQ ID NO: 10 - DNA, 46 bp, Artificial Sequence
  ra36428s01, primer allele X
gaaggtgaccaagttcatgctaatctctcaattgaaccgagaaccg

SEQ ID NO: 11 - DNA, 51 bp, Artificial Sequence
  ra74835s01, primer allele X
gaaggtgaccaagttcatgctaagcattgtggtccaaatataattcatgta

SEQ ID NO: 12 - DNA, 53 bp, Artificial Sequence
  ra74836s01, primer allele X
gaaggtgaccaagttcatgcttaaaagttaatttaaacatgtctgattaaaat

SEQ ID NO: 13 - DNA, 53 bp, Artificial Sequence
  ra74837s01, primer allele X
gaaggtgaccaagttcatgctaacgttatcgaatatcactgtaattaattgat

SEQ ID NO: 14 - DNA, 50 bp, Artificial Sequence
  ra74838s01, primer allele X
gaaggtgaccaagttcatgctgacaccaaactgattgatcaaaattgttc

SEQ ID NO: 15 - DNA, 54 bp, Artificial Sequence
  ra74840s01, primer allele X
gaaggtgaccaagttcatgctaataaaagtctggaccttttttttaacaaagtt

SEQ ID NO: 16 - DNA, 44 bp, Artificial Sequence
  ra74841s01, primer allele X
gaaggtgaccaagttcatgctcagtgtttctactaggagctgag

SEQ ID NO: 17 - DNA, 53 bp, Artificial Sequence
  ra74844s01, primer allele X
gaaggtgaccaagttcatgctaaaaataagatggaaatattgttgtgtaaaac

SEQ ID NO: 18 - DNA, 44 bp, Artificial Sequence
  ra74846s01, primer allele X
gaaggtgaccaagttcatgctgaacagacttggcaggtgagttg

SEQ ID NO: 19 - DNA, 47 bp, Artificial Sequence
  ra74847s01, primer allele X
gaaggtgaccaagttcatgctcatcataggtactatctcagctatgc

SEQ ID NO: 20 - DNA, 47 bp, Artificial Sequence
  ra74848s01, primer allele X
gaaggtgaccaagttcatgctatagcagacaataaagggttggtgtt

SEQ ID NO: 21 - DNA, 46 bp, Artificial Sequence
  ra74873s01, primer allele X
gaaggtgaccaagttcatgcttgtgaaagatgcaagaagaaagagg

SEQ ID NO: 22 - DNA, 43 bp, Artificial Sequence
  ra74851s01, primer allele X
gaaggtgaccaagttcatgctcctaagacctactggccgtaca

SEQ ID NO: 23 - DNA, 46 bp, Artificial Sequence
  ra74852s01, primer allele X
gaaggtgaccaagttcatgctattttccactcccgcatgaaacaca

SEQ ID NO: 24 - DNA, 44 bp, Artificial Sequence
  ra74854s01, primer allele X
gaaggtgaccaagttcatgctgggaacgagttgatgaagctgga

SEQ ID NO: 25 - DNA, 50 bp, Artificial Sequence
  ra74855s01, primer allele X
gaaggtgaccaagttcatgctactgactatttgtcttaaagtcaactatg

SEQ ID NO: 26 - DNA, 51 bp, Artificial Sequence
  ra74856s01, primer allele X
gaaggtgaccaagttcatgctgtatttctttctcctaccaagtttgattta

SEQ ID NO: 27 - DNA, 44 bp, Artificial Sequence
  ra74858s01, primer allele X
gaaggtgaccaagttcatgctgagctccgatgagagaaagcagt

SEQ ID NO: 28 - DNA, 42 bp, Artificial Sequence
  ra74859s01, primer allele X
gaaggtgaccaagttcatgctagcctgacagttgatgacacc

SEQ ID NO: 29 - DNA, 44 bp, Artificial Sequence
  ra74860s01, primer allele X
gaaggtgaccaagttcatgctccctctctgttattgtccttgcg

SEQ ID NO: 30 - DNA, 49 bp, Artificial Sequence
  ra74862s01, primer allele X
gaaggtgaccaagttcatgctgtacaggtttgattgcttgtcttctttt

SEQ ID NO: 31 - DNA, 51 bp, Artificial Sequence
  ra74863s01, primer allele X
gaaggtgaccaagttcatgctgcaaccagtaatttttttgtcttgagaata

SEQ ID NO: 32 - DNA, 51 bp, Artificial Sequence
  ra74864s01, primer allele X
gaaggtgaccaagttcatgcttagagaaaatatcatcaaaacaaatagcat

SEQ ID NO: 33 - DNA, 42 bp, Artificial Sequence
  ra74865s01, primer allele X
gaaggtgaccaagttcatgctccaaatctccacgagtgcagc

SEQ ID NO: 34 - DNA, 46 bp, Artificial Sequence
  ra74867s01, primer allele X
gaaggtgaccaagttcatgctatctggtgatcaagagcggttagtt

SEQ ID NO: 35 - DNA, 52 bp, Artificial Sequence
  ra74869s01, primer allele X
gaaggtgaccaagttcatgctataagtcccaatttttgataaaagaacaatc

SEQ ID NO: 36 - DNA, 44 bp, Artificial Sequence
  ra74870s01, primer allele X
gaaggtgaccaagttcatgcttcacctctcaagtgattctcagc

SEQ ID NO: 37 - DNA, 44 bp, Artificial Sequence
  ra74871s01, primer allele X
gaaggtgaccaagttcatgctcatgggggcaatcaatcatacgg

SEQ ID NO: 38 - DNA, 44 bp, Artificial Sequence
  ra74915s01, primer allele X
gaaggtgaccaagttcatgctggtcaataaggaggagaggacag

SEQ ID NO: 39 - DNA, 46 bp, Artificial Sequence
  ra74916s01, primer allele X
gaaggtgaccaagttcatgctagaggagaaacgagaaaacgctttc

SEQ ID NO: 40 - DNA, 53 bp, Artificial Sequence
  ra74917s01, primer allele X
gaaggtgaccaagttcatgctattcaaatcttattctacaccattaatccaat

SEQ ID NO: 41 - DNA, 52 bp, Artificial Sequence
  ra74919s01, primer allele X
gaaggtgaccaagttcatgctatcaattttaggttcttgcttaacaactttt

SEQ ID NO: 42 - DNA, 45 bp, Artificial Sequence
  ra74921s01, primer allele X
gaaggtgaccaagttcatgctgtaacacacgaccttaatcgtcgt

SEQ ID NO: 43 - DNA, 45 bp, Artificial Sequence
  ra74922s01, primer allele X
gaaggtgaccaagttcatgctgggatgtaggtatttgtctctgca

SEQ ID NO: 44 - DNA, 47 bp, Artificial Sequence
  ra74938s01, primer allele X
gaaggtgaccaagttcatgctgtgacattaggtatgtcaccacatca

SEQ ID NO: 45 - DNA, 43 bp, Artificial Sequence
  ra74941s01, primer allele X
gaaggtgaccaagttcatgctgagaggaaatgaggcgtaactc

SEQ ID NO: 46 - DNA, 53 bp, Artificial Sequence
  ra74949s01, primer allele X
gaaggtgaccaagttcatgctgtacatatttgtatataaagaagtggtttctc

SEQ ID NO: 47 - DNA, 47 bp, Artificial Sequence
  ra74932s02, primer allele X
gaaggtgaccaagttcatgctcagagcagtttgagaaattgaaacag

SEQ ID NO: 48 - DNA, 54 bp, Artificial Sequence
  ra74955s01, primer allele X
gaaggtgaccaagttcatgctaatttaaaccaacatataagctctataaagagt

SEQ ID NO: 49 - DNA, 48 bp, Artificial Sequence
  ra74945s01, primer allele X
gaaggtgaccaagttcatgctagctggacatctgggaatctaaatata

SEQ ID NO: 50 - DNA, 49 bp, Artificial Sequence
  ra74946s01, primer allele X
gaaggtgaccaagttcatgctcatttcttaactcacacattgcttgtca

SEQ ID NO: 51 - DNA, 47 bp, Artificial Sequence
  ra74948s01, primer allele X
gaaggtgaccaagttcatgctggaggcatcttaagtatcccattatc

SEQ ID NO: 52 - DNA, 40 bp, Artificial Sequence
  ra74952s01, primer allele X
gaaggtgaccaagttcatgcttccctgagcggtgacagtc

SEQ ID NO: 53 - DNA, 49 bp, Artificial Sequence; identical to SEQ ID NO: 50
  ra74946s01, primer allele X

SEQ ID NO: 54 - DNA, 47 bp, Artificial Sequence; identical to SEQ ID NO: 51
  ra74948s01, primer allele X

SEQ ID NO: 55 - DNA, 40 bp, Artificial Sequence; identical to SEQ ID NO: 52
  ra74952s01, primer allele X

SEQ ID NO: 56 - DNA, 45 bp, Artificial Sequence
  ra01867s01, primer allele X
gaaggtgaccaagttcatgctataaagtagcaaaggagccagctg

SEQ ID NO: 57 - DNA, 51 bp, Artificial Sequence
  ra01868s01, primer allele X
gaaggtgaccaagttcatgctactacaaacaagtcaaatgcaaaatcagaa

SEQ ID NO: 58 - DNA, 46 bp, Artificial Sequence
  ra13870s01, primer allele X
gaaggtgaccaagttcatgctaagaggcatattgttctttggacat

SEQ ID NO: 59 - DNA, 42 bp, Artificial Sequence
  ra17237s01, primer allele X
gaaggtgaccaagttcatgctgcgatcctaaaccgggtagcc

SEQ ID NO: 60 - DNA, 51 bp, Artificial Sequence
  ra36486s01, primer allele X
gaaggtgaccaagttcatgctatcacttttktaagtttctttttaaatcac

SEQ ID NO: 61 - DNA, 44 bp, Artificial Sequence
  ra36162s01, primer allele X
gaaggtgaccaagttcatgctcccctttcattcgtacttaccgc

SEQ ID NO: 62 - DNA, 51 bp, Artificial Sequence
  ra36410s01, primer allele X
gaaggtgaccaagttcatgctcaaagttattttctgcagaatgtgagaatt

SEQ ID NO: 63 - DNA, 48 bp, Artificial Sequence
  ra36412s01, primer allele X
gaaggtgaccaagttcatgctttcactccaatctrttgacatgataac

SEQ ID NO: 64 - DNA, 47 bp, Artificial Sequence
  ra36483s01, primer allele X
gaaggtgaccaagttcatgctgtggaaacagagaagaaactcatgag

SEQ ID NO: 65 - DNA, 50 bp, Artificial Sequence
  ra74872s01, primer allele X
gaaggtgaccaagttcatgctgaaaagatcattacttcactccaagtaag

SEQ ID NO: 66 - DNA, 46 bp, Artificial Sequence
  ra74910s01, primer allele X
gaaggtgaccaagttcatgctagtcctgacacccagattggtaaat

SEQ ID NO: 67 - DNA, 45 bp, Artificial Sequence
  ra74958s01, primer allele X
gaaggtgaccaagttcatgctactctctcactacctcgaaaatgg

SEQ ID NO: 68 - DNA, 50 bp, Artificial Sequence
  ra74958s02, primer allele X
gaaggtgaccaagttcatgctcattgggaatattcttcatatgtttggca

SEQ ID NO: 69 - DNA, 49 bp, Artificial Sequence
  ra74958s03, primer allele X
gaaggtgaccaagttcatgctgtatcattaagctgtagactatagttta

SEQ ID NO: 70 - DNA, 51 bp, Artificial Sequence
  ra74958s04, primer allele X
gaaggtgaccaagttcatgctcatcactaattgaaatgcattcattagaac

SEQ ID NO: 71 - DNA, 47 bp, Artificial Sequence
  ra74958s05, primer allele X
gaaggtgaccaagttcatgcttgttgtttcttttgtagcaagctgct

SEQ ID NO: 72 - DNA, 50 bp, Artificial Sequence
  ra74958s06, primer allele X
gaaggtgaccaagttcatgctgaaacaacaatggtttaaaggcgcaatta

SEQ ID NO: 73 - DNA, 48 bp, Artificial Sequence
  ra74958s07, primer allele X
gaaggtgaccaagttcatgctgtttaaaggcgcaattmtcaaggtgaa

SEQ ID NO: 74 - DNA, 49 bp, Artificial Sequence
  ra74958s08, primer allele X
gaaggtgaccaagttcatgctgaatcccttatgaatttttgttactacg

SEQ ID NO: 75 - DNA, 45 bp, Artificial Sequence
  ra36387s01, primer allele Y
gaaggtcggagtcaacggattaatcggagacgaatttggagtggt

SEQ ID NO: 76 - DNA, 50 bp, Artificial Sequence
  ra36444s01, primer allele Y
gaaggtcggagtcaacggattcaatgcttcaagtaacacatttagaaaca

SEQ ID NO: 77 - DNA, 52 bp, Artificial Sequence
  ra36450s01, primer allele Y
gaaggtcggagtcaacggattattayaatgactatgaattttgctaaccatg

SEQ ID NO: 78 - DNA, 41 bp, Artificial Sequence
  ra36451s01, primer allele Y
gaaggtcggagtcaacggattctgcgggaggagagcttctg

SEQ ID NO: 79 - DNA, 48 bp, Artificial Sequence
  ra36458s01, primer allele Y
gaaggtcggagtcaacggattgattgarttcattctgttttcggtttg

SEQ ID NO: 80 - DNA, 44 bp, Artificial Sequence
  ra36459s01, primer allele Y
gaaggtcggagtcaacggattggtggttacaagataaggtaccg

SEQ ID NO: 81 - DNA, 48 bp, Artificial Sequence
  ra36460s01, primer allele Y
gaaggtcggagtcaacggattaacaaagatttccacgccaaaattctg

SEQ ID NO: 82 - DNA, 47 bp, Artificial Sequence
  ra36461s01, primer allele Y
gaaggtcggagtcaacggattatcggacactctacatctttaagttc

SEQ ID NO: 83 - DNA, 51 bp, Artificial Sequence
  ra36463s01, primer allele Y
gaaggtcggagtcaacggattaatataggaacttatgaatctaacgttcca

SEQ ID NO: 84 - DNA, 46 bp, Artificial Sequence
  ra36428s01, primer allele Y
gaaggtcggagtcaacggattaatctctcaattgaaccgagaacca

SEQ ID NO: 85 - DNA, 49 bp, Artificial Sequence
  ra74835s01, primer allele Y
gaaggtcggagtcaacggattgcattgtggtccaaatataattcatgtg

SEQ ID NO: 86 - DNA, 52 bp, Artificial Sequence
  ra74836s01, primer allele Y
gaaggtcggagtcaacggattaaaagttaatttaaacatgtctgattaaaaa

SEQ ID NO: 87 - DNA, 51 bp, Artificial Sequence
  ra74837s01, primer allele Y
gaaggtcggagtcaacggattcgttatcgaatatcactgtaattaattgag

SEQ ID NO: 88 - DNA, 50 bp, Artificial Sequence
  ra74838s01, primer allele Y
gaaggtcggagtcaacggattgacaccaaactgattgatcaaaattgttt

SEQ ID NO: 89 - DNA, 51 bp, Artificial Sequence
  ra74840s01, primer allele Y
gaaggtcggagtcaacggattaaaagtctggaccttttttttaacaaagtg

SEQ ID NO: 90 - DNA, 45 bp, Artificial Sequence
  ra74841s01, primer allele Y
gaaggtcggagtcaacggattgcagtgtttctactaggagctgaa

SEQ ID NO: 91 - DNA, 53 bp, Artificial Sequence
  ra74844s01, primer allele Y
gaaggtcggagtcaacggattaaaaataagatggaaatattgttgtgtaaaag

SEQ ID NO: 92 - DNA, 44 bp, Artificial Sequence
  ra74846s01, primer allele Y
gaaggtcggagtcaacggattgaacagacttggcaggtgagtta

SEQ ID NO: 93 - DNA, 47 bp, Artificial Sequence
  ra74847s01, primer allele Y
gaaggtcggagtcaacggattcatcataggtactatctcagctatgt

SEQ ID NO: 94 - DNA, 45 bp, Artificial Sequence
  ra74848s01, primer allele Y
gaaggtcggagtcaacggattagcagacaataaagggttggtgtc

SEQ ID NO: 95 - DNA, 48 bp, Artificial Sequence
  ra74873s01, primer allele Y
gaaggtcggagtcaacggattcttgtgaaagatgcaagaagaaagaga

SEQ ID NO: 96 - DNA, 42 bp, Artificial Sequence
  ra74851s01, primer allele Y
gaaggtcggagtcaacggattctaagacctactggccgtacg

SEQ ID NO: 97 - DNA, 41 bp, Artificial Sequence
  ra74852s01, primer allele Y
gaaggtcggagtcaacggattccactcccgcatgaaacacg

SEQ ID NO: 98 - DNA, 44 bp, Artificial Sequence
  ra74854s01, primer allele Y
gaaggtcggagtcaacggattgggaacgagttgatgaagctggt

SEQ ID NO: 99 - DNA, 52 bp, Artificial Sequence
  ra74855s01, primer allele Y
gaaggtcggagtcaacggattgtactgactatttgtcttaaagtcaactata

SEQ ID NO: 100 - DNA, 49 bp, Artificial Sequence
  ra74856s01, primer allele Y
gaaggtcggagtcaacggattatttctttctcctaccaagtttgatttc

SEQ ID NO: 101 - DNA, 44 bp, Artificial Sequence
  ra74858s01, primer allele Y
gaaggtcggagtcaacggattgagctccgatgagagaaagcaga

SEQ ID NO: 102 - DNA, 46 bp, Artificial Sequence
  ra74859s01, primer allele Y
gaaggtcggagtcaacggattaactagcctgacagttgatgacact

SEQ ID NO: 103 - DNA, 46 bp, Artificial Sequence
  ra74860s01, primer allele Y
gaaggtcggagtcaacggattaaccctctctgttattgtccttgct

SEQ ID NO: 104 - DNA, 49 bp, Artificial Sequence
  ra74862s01, primer allele Y
gaaggtcggagtcaacggattgtacaggtttgattgcttgtcttcttta

SEQ ID NO: 105 - DNA, 50 bp, Artificial Sequence
  ra74863s01, primer allele Y
gaaggtcggagtcaacggattcaaccagtaatttttttgtcttgagaatc

SEQ ID NO: 106 - DNA, 53 bp, Artificial Sequence
  ra74864s01, primer allele Y
gaaggtcggagtcaacggattcttagagaaaatatcatcaaaacaaatagcag

SEQ ID NO: 107 - DNA, 44 bp, Artificial Sequence
  ra74865s01, primer allele Y
gaaggtcggagtcaacggattctccaaatctccacgagtgcagt

SEQ ID NO: 108 - DNA, 44 bp, Artificial Sequence
  ra74867s01, primer allele Y
gaaggtcggagtcaacggattctggtgatcaagagcggttagtg

SEQ ID NO: 109 - DNA, 54 bp, Artificial Sequence
  ra74869s01, primer allele Y
gaaggtcggagtcaacggattctataagtcccaatttttgataaaagaacaatt

SEQ ID NO: 110 - DNA, 46 bp, Artificial Sequence
  ra74870s01, primer allele Y
gaaggtcggagtcaacggattcttcacctctcaagtgattctcaga

SEQ ID NO: 111 - DNA, 45 bp, Artificial Sequence
  ra74871s01, primer allele Y
gaaggtcggagtcaacggattacatgggggcaatcaatcatacgt

SEQ ID NO: 112 - DNA, 44 bp, Artificial Sequence
  ra74915s01, primer allele Y
gaaggtcggagtcaacggattggtcaataaggaggagaggacat

SEQ ID NO: 113 - DNA, 46 bp, Artificial Sequence
  ra74916s01, primer allele Y
gaaggtcggagtcaacggattagaggagaaacgagaaaacgcttta

SEQ ID NO: 114 - DNA, 50 bp, Artificial Sequence
  ra74917s01, primer allele Y
gaaggtcggagtcaacggattcaaatcttattctacaccattaatccaac

SEQ ID NO: 115 - DNA, 50 bp, Artificial Sequence
  ra74919s01, primer allele Y
gaaggtcggagtcaacggattcaattttaggttcttgcttaacaactttc

SEQ ID NO: 116 - DNA, 43 bp, Artificial Sequence
  ra74921s01, primer allele Y
gaaggtcggagtcaacggattaacacacgaccttaatcgtcgc

SEQ ID NO: 117 - DNA, 44 bp, Artificial Sequence
  ra74922s01, primer allele Y
gaaggtcggagtcaacggattggatgtaggtatttgtctctgcg

SEQ ID NO: 118 - DNA, 45 bp, Artificial Sequence
  ra74938s01, primer allele Y
gaaggtcggagtcaacggattgacattaggtatgtcaccacatcg

SEQ ID NO: 119 - DNA, 46 bp, Artificial Sequence
  ra74941s01, primer allele Y
gaaggtcggagtcaacggattagtgagaggaaatgaggcgtaacta

SEQ ID NO: 120 - DNA, 53 bp, Artificial Sequence
  ra74949s01, primer allele Y
gaaggtcggagtcaacggattgtacatatttgtatataaagaagtggtttcta

SEQ ID NO: 121 - DNA, 50 bp, Artificial Sequence
  ra74932s02, primer allele Y
gaaggtcggagtcaacggattgatcagagcagtttgagaaattgaaacaa

SEQ ID NO: 122 - DNA, 54 bp, Artificial Sequence
  ra74955s01, primer allele Y
gaaggtcggagtcaacggattaatttaaaccaacatataagctctataaagaga

SEQ ID NO: 123 - DNA, 47 bp, Artificial Sequence
  ra74945s01, primer allele Y
gaaggtcggagtcaacggattgctggacatctgggaatctaaatatc

SEQ ID NO: 124 - DNA, 45 bp, Artificial Sequence
  ra74946s01, primer allele Y
gaaggtcggagtcaacggatttcttaactcacacattgcttgtcg

SEQ ID NO: 125 - DNA, 47 bp, Artificial Sequence
  ra74948s01, primer allele Y
gaaggtcggagtcaacggattggaggcatcttaagtatcccattata

SEQ ID NO: 126 - DNA, 42 bp, Artificial Sequence
  ra74952s01, primer allele Y
gaaggtcggagtcaacggattcttccctgagcggtgacagtt

SEQ ID NO: 127 - DNA, 46 bp, Artificial Sequence
  ra01867s01, primer allele Y
gaaggtcggagtcaacggattcataaagtagcaaaggagccagctt

SEQ ID NO: 128 - DNA, 50 bp, Artificial Sequence
  ra01868s01, primer allele Y
gaaggtcggagtcaacggattctacaaacaagtcaaatgcaaaatcagac

SEQ ID NO: 129 - DNA, 46 bp, Artificial Sequence
  ra13870s01, primer allele Y
gaaggtcggagtcaacggattaagaggcatattgttctttggacac

SEQ ID NO: 130 - DNA, 43 bp, Artificial Sequence
  ra17237s01, primer allele Y
gaaggtcggagtcaacggattagcgatcctaaaccgggtagca

SEQ ID NO: 131 - DNA, 53 bp, Artificial Sequence
  ra36486s01, primer allele Y
gaaggtcggagtcaacggattctatcacttttktaagtttctttttaaatcaa

SEQ ID NO: 132 - DNA, 46 bp, Artificial Sequence
  ra36162s01, primer allele Y
gaaggtcggagtcaacggattatcccctttcattcgtacttaccgt

SEQ ID NO: 133 - DNA, 50 bp, Artificial Sequence
  ra36410s01, primer allele Y
gaaggtcggagtcaacggattaaagttattttctgcagaatgtgagaatc

SEQ ID NO: 134 - DNA, 49 bp, Artificial Sequence
  ra36412s01, primer allele Y
gaaggtcggagtcaacggatttttcactccaatctrttgacatgataat

SEQ ID NO: 135 - DNA, 47 bp, Artificial Sequence
  ra36483s01, primer allele Y
gaaggtcggagtcaacggattgtggaaacagagaagaaactcatgaa

SEQ ID NO: 136 - DNA, 50 bp, Artificial Sequence
  ra74872s01, primer allele Y
gaaggtcggagtcaacggattgaaaagatcattacttcactccaagtaaa

SEQ ID NO: 137 - DNA, 43 bp, Artificial Sequence
  ra74910s01, primer allele Y
gaaggtcggagtcaacggattcctgacacccagattggtaaac

SEQ ID NO: 138 - DNA, 46 bp, Artificial Sequence
  ra74958s01, primer allele Y
gaaggtcggagtcaacggattcactctctcactacctcgaaaatga

SEQ ID NO: 139 - DNA, 50 bp, Artificial Sequence
  ra74958s02, primer allele Y
gaaggtcggagtcaacggattcattgggaatattcttcatatgtttggct

SEQ ID NO: 140 - DNA, 49 bp, Artificial Sequence
  ra74958s03, primer allele Y
gaaggtcggagtcaacggattgtatcattaagctgtagactatagtttg

SEQ ID NO: 141 - DNA, 51 bp, Artificial Sequence
  ra74958s04, primer allele Y
gaaggtcggagtcaacggattcatcactaattgaaatgcattcattagaag

SEQ ID NO: 142 - DNA, 46 bp, Artificial Sequence
  ra74958s05, primer allele Y
gaaggtcggagtcaacggattgttgtttcttttgtagcaagctgcg

SEQ ID NO: 143 - DNA, 48 bp, Artificial Sequence
  ra74958s06, primer allele Y
gaaggtcggagtcaacggattaacaacaatggtttaaaggcgcaattc

SEQ ID NO: 144 - DNA, 45 bp, Artificial Sequence
  ra74958s07, primer allele Y
gaaggtcggagtcaacggatttaaaggcgcaattmtcaaggtgac

SEQ ID NO: 145 - DNA, 49 bp, Artificial Sequence
  ra74958s08, primer allele Y
gaaggtcggagtcaacggattgaatcccttatgaatttttgttactacc

SEQ ID NO: 146 - DNA, 26 bp, Artificial Sequence
  ra36387s01, common primer
ggcggaaacaacagcttcaaactgtt

SEQ ID NO: 147 - DNA, 24 bp, Artificial Sequence
  ra36444s01, common primer
cttccggcgttggaatcactgaaa

SEQ ID NO: 148 - DNA, 29 bp, Artificial Sequence
  ra36450s01, common primer
gtaggaaccctgtaagaatagattctcaa

SEQ ID NO: 149 - DNA, 29 bp, Artificial Sequence
  ra36451s01, common primer
tcgtgttatcttgtaaaccgtacctagtt

SEQ ID NO: 150 - DNA, 28 bp, Artificial Sequence
  ra36458s01, common primer
gccaagccttgtagagttacaaagatat

SEQ ID NO: 151 - DNA, 29 bp, Artificial Sequence
  ra36459s01, common primer
gaaacctgaagagtaagtcagttagacaa

SEQ ID NO: 152 - DNA, 26 bp, Artificial Sequence
  ra36460s01, common primer
ggtgccttgattcttctcttcctctt

SEQ ID NO: 153 - DNA, 30 bp, Artificial Sequence
  ra36461s01, common primer
caaaggtaaaaatggttcatggttgctgtt

SEQ ID NO: 154 - DNA, 30 bp, Artificial Sequence
  ra36463s01, common primer
gccttttcaaaatattcttttgcctacatt

SEQ ID NO: 155 - DNA, 30 bp, Artificial Sequence
  ra36428s01, common primer
gaaacaacattgttgagctacaatctctta

SEQ ID NO: 156 - DNA, 25 bp, Artificial Sequence
  ra74835s01, common primer
gttattggtgcatgggtgccaagta

SEQ ID NO: 157 - DNA, 29 bp, Artificial Sequence
  ra74836s01, common primer
tgatcggacttctcaaagtttgtaccttt

SEQ ID NO: 158 - DNA, 29 bp, Artificial Sequence
  ra74837s01, common primer
gactagaacatccaacaaatgagagcatt

SEQ ID NO: 159 - DNA, 29 bp, Artificial Sequence
  ra74838s01, common primer
tctttttcagatcgcacgttgtgtgaaat

SEQ ID NO: 160 - DNA, 29 bp, Artificial Sequence
  ra74840s01, common primer
acacgtatgagaagccaaataacggtaaa

SEQ ID NO: 161 - DNA, 29 bp, Artificial Sequence
  ra74841s01, common primer
gggatgttttgtcaaacaaagaagctgtt

SEQ ID NO: 162 - DNA, 30 bp, Artificial Sequence
  ra74844s01, common primer
gacactcatttgaaatctttgtggatgaat

SEQ ID NO: 163 - DNA, 25 bp, Artificial Sequence
  ra74846s01, common primer
gccacaagtcacatgaccacaactt

SEQ ID NO: 164 - DNA, 28 bp, Artificial Sequence
  ra74847s01, common primer
atctccgggattttatttcgttgcagtt

SEQ ID NO: 165 - DNA, 30 bp, Artificial Sequence
  ra74848s01, common primer
gagtctatgtaacaagatgtttaatctaat

SEQ ID NO: 166 - DNA, 29 bp, Artificial Sequence
  ra74873s01, common primer
aacatgtatggtctcttcactggtatgat

SEQ ID NO: 167 - DNA, 28 bp, Artificial Sequence
  ra74851s01, common primer
ggtttatgagaatgactgcagtagcaaa

SEQ ID NO: 168 - DNA, 29 bp, Artificial Sequence
  ra74852s01, common primer
cacgttgttgcgtatgaaatgatagtcta

SEQ ID NO: 169 - DNA, 30 bp, Artificial Sequence
  ra74854s01, common primer
gattaagaaacaacaaacctgtacaggtat

SEQ ID NO: 170 - DNA, 29 bp, Artificial Sequence
  ra74855s01, common primer
cgaagcaagtttcttgtgatcttgtcaat

SEQ ID NO: 171 - DNA, 30 bp, Artificial Sequence
  ra74856s01, common primer
tgtgggtgatgaaaaagaaagaaagagata

SEQ ID NO: 172 - DNA, 30 bp, Artificial Sequence
  ra74858s01, common primer
ctccagagaaaataatattctcgttctcca

SEQ ID NO: 173 - DNA, 29 bp, Artificial Sequence
  ra74859s01, common primer
tcactatcttgacctccaagaatcagttt

SEQ ID NO: 174 - DNA, 26 bp, Artificial Sequence
  ra74860s01, common primer
gaaacagaggatcaggtgaaagcgaa

SEQ ID NO: 175 - DNA, 29 bp, Artificial Sequence
  ra74862s01, common primer
cacgcatgtcaatggttcatctcttatat

SEQ ID NO: 176 - DNA, 29 bp, Artificial Sequence
  ra74863s01, common primer
gtcatgtttagtgcctaccaaaatgctaa

SEQ ID NO: 177 - DNA, 30 bp, Artificial Sequence
  ra74864s01, common primer
ctcaaaaagtaaatttgatgtttgtgttat

SEQ ID NO: 178 - DNA, 25 bp, Artificial Sequence
  ra74865s01, common primer
ggtgaagaccatgtggagtcaagat

SEQ ID NO: 179 - DNA, 25 bp, Artificial Sequence
  ra74867s01, common primer
atgactccgctgctcttccaagata

SEQ ID NO: 180 - DNA, 29 bp, Artificial Sequence
  ra74869s01, common primer
cttctagctttgatcatttcttcgtcact

SEQ ID NO: 181 - DNA, 28 bp, Artificial Sequence
  ra74870s01, common primer
aaacttgtcccgtctcacaaatcttctt

SEQ ID NO: 182 - DNA, 30 bp, Artificial Sequence
  ra74871s01, common primer
ctacacctttatacatcatatccatcgaat

SEQ ID NO: 183 - DNA, 28 bp, Artificial Sequence
  ra74915s01, common primer
ccttctccagtattcattagagtgagtt

SEQ ID NO: 184 - DNA, 23 bp, Artificial Sequence
  ra74916s01, common primer
cgtcgtacggccattctcaggta

SEQ ID NO: 185 - DNA, 30 bp, Artificial Sequence
  ra74917s01, common primer
kcatttttattccgtttgattccttgagaa

SEQ ID NO: 186 - DNA, 22 bp, Artificial Sequence
  ra74919s01, common primer
gagcgtgtggcgtaagggagat

SEQ ID NO: 187 - DNA, 28 bp, Artificial Sequence
  ra74921s01, common primer
gttctcattacctatacacacgttcctt

SEQ ID NO: 188 - DNA, 30 bp, Artificial Sequence
  ra74922s01, common primer
gtctacaacacttttttaaactcatgtctt

SEQ ID NO: 189 - DNA, 27 bp, Artificial Sequence
  ra74938s01, common primer
caggaatatactaaagggctccaggaa

SEQ ID NO: 190 - DNA, 29 bp, Artificial Sequence
  ra74941s01, common primer
gagagtcagtgttataaaacgacacgata

SEQ ID NO: 191 - DNA, 30 bp, Artificial Sequence
  ra74949s01, common primer
cagaatcttgcattgctacagatactagaa

SEQ ID NO: 192 - DNA, 22 bp, Artificial Sequence
  ra74932s02, common primer
ttcgctccaccgctgccttgaa

SEQ ID NO: 193 - DNA, 27 bp, Artificial Sequence
  ra74955s01, common primer
tgaaggtatgctttatcctcctcagtt

SEQ ID NO: 194 - DNA, 29 bp, Artificial Sequence
  ra74945s01, common primer
gactatcaaattgatgttccaccagtctt

SEQ ID NO: 195 - DNA, 29 bp, Artificial Sequence
  ra74946s01, common primer
caactgagaacttgattcctgatccaaat

SEQ ID NO: 196 - DNA, 29 bp, Artificial Sequence
  ra74948s01, common primer
gttcgtcatcttgatgttcgtaatgagtt

SEQ ID NO: 197 - DNA, 25 bp, Artificial Sequence
  ra74952s01, common primer
cagcataaatgacggcgaggaagta

SEQ ID NO: 198 - DNA, 25 bp, Artificial Sequence
  ra01867s01, common primer
actctcgctctactccatcagcttt

SEQ ID NO: 199 - DNA, 29 bp, Artificial Sequence
  ra01868s01, common primer
ctcctttgctactttatgttcttctccat

SEQ ID NO: 200 - DNA, 30 bp, Artificial Sequence
  ra13870s01, common primer
gtcawagaaacaaggctgagaatatcagtt

SEQ ID NO: 201 - DNA, 25 bp, Artificial Sequence
  ra17237s01, common primer
ctagcttccctcgtagacaccttat

SEQ ID NO: 202 - DNA, 30 bp, Artificial Sequence
  ra36486s01, common primer
cggagatataaaaaatgataccaatagcat

SEQ ID NO: 203 - DNA, 30 bp, Artificial Sequence
  ra36162s01, common primer
gaccratattagttagttatyaaatccttt

SEQ ID NO: 204 - DNA, 22 bp, Artificial Sequence
  ra36410s01, common primer
ccactgatccttccaacrttca

SEQ ID NO: 205 - DNA, 30 bp, Artificial Sequence
  ra36412s01, common primer
cagaactgttccatgagaaactattcagta

SEQ ID NO: 206 - DNA, 24 bp, Artificial Sequence
  ra36483s01, common primer
actttggcctmctctgtgctcact

SEQ ID NO: 207 - DNA, 30 bp, Artificial Sequence
  ra74872s01, common primer
agcaaaaatatcacctaatgaggaataata

SEQ ID NO: 208 - DNA, 25 bp, Artificial Sequence
  ra74910s01, common primer
agaaagctgtggtcacaactgcctt

SEQ ID NO: 209 - DNA, 30 bp, Artificial Sequence
  ra74958s01, common primer
gggttttaaattctcttgcttctttctcct

SEQ ID NO: 210 - DNA, 30 bp, Artificial Sequence
  ra74958s02, common primer
tccccaaaatagtcaaatgattacacgatt

SEQ ID NO: 211 - DNA, 28 bp, Artificial Sequence
  ra74958s03, common primer
gaaattcttctgacattcatcagagtgc

SEQ ID NO: 212 - DNA, 29 bp, Artificial Sequence
  ra74958s04, common primer
gcactagatgataagattctggtactgtt

SEQ ID NO: 213 - DNA, 25 bp, Artificial Sequence
  ra74958s05, common primer
ctcctctggatgtagatcctctagt

SEQ ID NO: 214 - DNA, 29 bp, Artificial Sequence
  ra74958s06, common primer
gtggatcgtctttggttaacttaatgcat

SEQ ID NO: 215 - DNA, 25 bp, Artificial Sequence
  ra74958s07, common primer
cgtggtaagtggatcgtctttggtt

SEQ ID NO: 216 - DNA, 26 bp, Artificial Sequence
  ra74958s08, common primer
gggcaccaactaacctaaagagagtt

SEQ ID NO: 217 - DNA, 25 bp, Artificial Sequence
  ra74958s05, common primer
ctcctctggatgtagatcctctagt

SEQ ID NO: 218 - DNA, 29 bp, Artificial Sequence
  ra74958s06, common primer
gtggatcgtctttggttaacttaatgcat

SEQ ID NO: 219 - DNA, 25 bp, Artificial Sequence
  ra74958s07, common primer
cgtggtaagtggatcgtctttggtt

SEQ ID NO: 220 - DNA, 26 bp, Artificial Sequence
  ra74958s08, common primer
gggcaccaactaacctaaagagagtt

SEQ ID NO: 221 - DNA, 26 bp, Artificial Sequence
  ra74958s08, common primer
gggcaccaactaacctaaagagagtt

SEQ ID NO: 222 - DNA, 101 bp, Artificial Sequence
  ra36387s01, marker
ctttggaggtytgggcttgtgtgaaggaatcggagacgaatttggagtggyagcaacagtttgaagctgttgtttccgccaggatgtcatatcttcaacac

SEQ ID NO: 223 - DNA, 101 bp, Artificial Sequence
  ra36444s01, marker
agaaagtctcattatactttgcttcccttccggcgttggaatcactgaaaygtttctaaatgtgttacttgaagcattgatttagatattgaaccttgaac

SEQ ID NO: 224 - DNA, 101 bp, Artificial Sequence
  ra36450s01, marker
atttgaatctagtttaatatattayaatgactatgaattttgctaaccatrtgttgagaatctattcttacagggttcctacaactctgcgagtgttttcc

SEQ ID NO: 225 - DNA, 101 bp, Artificial Sequence
  ra36451s01, marker
cgtgttatcttgtaaaccgtacctagttcagaacgtgcaagacgaatggamagaagctctcctcccgcagaaaatttcaccacgtctattagctcstgact

SEQ ID NO: 226 - DNA, 101 bp, Artificial Sequence
  ra36458s01, marker
agtctggtgagtctcrcgagcattgattgarttcattctgttttcggtttrcatatctttgtaactctacaaggcttggcgtgtgaactaatgagctttct

SEQ ID NO: 227 - DNA, 101 bp, Artificial Sequence
  ra36459s01, marker
gagatttcgttgctcactgataaaatcgggtggttacaagataaggtaccrcaattgtctaactgacttactcttcaggtttcatatggaattattattct

SEQ ID NO: 228 - DNA, 101 bp, Artificial Sequence
  ra36460s01, marker
accatyattctcatacccaattagaacaaagatttccacgccaaaattctraaaagaggaagagaagaatcaaggcaccttgtttacgagatttcctcttc

SEQ ID NO: 229 - DNA, 101 bp, Artificial Sequence
  ra36461s01, marker
aaagcttggttgaagctttctttgcatcggacactctacatctttaagttmcaacagcaaccatgaaccatttttacctttgtamattccagctaattaaa

SEQ ID NO: 230 - DNA, 101 bp, Artificial Sequence
  ra36463s01, marker
aacagccttttcaaaatattcttttgcctacatttgamgccayattacaayggaacgttagattcataagttcctatattatatccatcgtctaaatatgt

SEQ ID NO: 231 - DNA, 101 bp, Artificial Sequence
  ra36428s01, marker
tcctctttccatgaaacaacattgttgagctacaatctcttagcaccggcyggttctcggttcaattgagagattagtttgatagaaaaccttccacggtg

SEQ ID NO: 232 - DNA, 101 bp, Artificial Sequence
  ra74835s01, marker
aaggttcatcatatcattatcaagcattgtggtccaaatataattcatgtrtattatatacttggcacccatgcaccaataacgcgtagtaaccacatagt

SEQ ID NO: 233 - DNA, 101 bp, Artificial Sequence
  ra74836s01, marker
acttctcaaagtttgtaccttttaaaaaaaaaacctttttgttgttctgtwttttaatcagacatgtttaaattaacttttaaatgttacagggaaggtac

SEQ ID NO: 234 - DNA, 101 bp, Artificial Sequence
  ra74837s01, marker
gaaaaagactagaacatccaacaaatgagagcattaaaagatctgaatttmtcaattaattacagtgatattcgataacgttgaaaaaagtgaatgatttt

SEQ ID NO: 235 - DNA, 101 bp, Artificial Sequence
  ra74838s01, marker
ttattaaagtaagagagagtacgacaccaaactgattgatcaaaattgttygagatttcacacaacgtgcgatctgaaaaagacagaaagaggcagagatg

SEQ ID NO: 236 - DNA, 101 bp, Artificial Sequence
  ra74840s01, marker
gtttgagctttgtacacgtatgagaagccaaataacggtaaaacgtttgamactttgttaaaaaaaaggtccagacttttattagtgaaaagtctgcgtat

SEQ ID NO: 237 - DNA, 101 bp, Artificial Sequence
  ra74841s01, marker
tgctaggtgtgggatgttttgtcaaacaaagaagctgttgatattgtggcytcagctcctagtagaaacactgcggctcgtgctttagtatgcacagctgt

SEQ ID NO: 238 - DNA, 101 bp, Artificial Sequence
  ra74844s01, marker
tgtgatgtaagaaactgttaaaaataagatggaaatattgttgtgtaaaastaaagaatattttgctattcatccacaaagatttcaaatgagtgtctata

SEQ ID NO: 239 - DNA, 101 bp, Artificial Sequence
  ra74846s01, marker
ctaaccaagtcttctagccacaagtcacatgaccacaacttacctgaccayaactcacctgccaagtctgttcacagctctcctgaccaagtcattgctga

SEQ ID NO: 240 - DNA, 101 bp, Artificial Sequence
  ra74847s01, marker
gcaaaagacatgtcacgactcatatcatcataggtactatctcagctatgyaactgcaacgaaataaaatcccggagatgtcaaaggtagcccaaaaaaca

SEQ ID NO: 241 - DNA, 101 bp, Artificial Sequence
  ra74848s01, marker
tatatcagtttatttatttgagtctatgtaacaagatgtttaatctaatgracaccaaccctttattgtctgctataaatgataaatccttgtttagaacg

SEQ ID NO: 242 - DNA, 101 bp, Artificial Sequence
  ra74873s01, marker
ctgtctttttcttgcaaaacatgtatggtctcttcactggtatgatgaccyctctttcttcttgcatctttcacaagatgctgctggcagcattggacaca

SEQ ID NO: 243 - DNA, 101 bp, Artificial Sequence
  ra74851s01, marker
gtctcacattgctcagccaagcggcggttcctaagacctactggccgtacrcttttgctactgcagtcattctcataaaccgactaccctctcccgtgctc

SEQ ID NO: 244 - DNA, 101 bp, Artificial Sequence
  ra74852s01, marker
gtgccacttacttgtgtgcgaatcccattttccactcccgcatgaaacacrtcgcgttagactatcatttcatacgcaacaacgtgcaatcgggggctctg

SEQ ID NO: 245 - DNA, 101 bp, Artificial Sequence
  ra74854s01, marker
caggtacgagctttatttgatcacagtggggaacgagttgatgaagctggwccctccatacctgtacaggtttgttgtttcttaatcttcctttaaagtca

SEQ ID NO: 246 - DNA, 101 bp, Artificial Sequence
  ra74855s01, marker
tcagacaagagtcaccagacgaagcaagtttcttgtgatcttgtcaatacyatagttgactttaagacaaatagtcagtaccttaattaatttaatcgttt

SEQ ID NO: 247 - DNA, 101 bp, Artificial Sequence
  ra74856s01, marker
ttgtaaaggtccttgtttcttgtatttctttctcctaccaagtttgatttmtatctctttctttctttttcatcacccacaaaaagttgattttgtttgtt

SEQ ID NO: 248 - DNA, 101 bp, Artificial Sequence
  ra74858s01, marker
tatagctaaaaataatcaatctccagagaaaataatattctcgttctccawctgctttctctcatcggagctctctttttctggttctcaaggtaagacaa

SEQ ID NO: 249 - DNA, 101 bp, Artificial Sequence
  ra74859s01, marker
cggattaacccatgtgttatcccaacaactagcctgacagttgatgacacyaaactgattcttggaggtcaagatagtgatatggttgttgcttttagcaa

SEQ ID NO: 250 - DNA, 101 bp, Artificial Sequence
  ra74860s01, marker
ttcaactttttgtgtgtgattcatgaaaccctctctgttattgtccttgckcttcgctttcacctgatcctctgtttctgtttttggataaagttcctaaa

SEQ ID NO: 251 - DNA, 101 bp, Artificial Sequence
  ra74862s01, marker
acgcatgtcaatggttcatctcttatataagatagagaagtactgaattgwaaagaagacaagcaatcaaacctgtacgagcctgttgctacccttgatcc

SEQ ID NO: 252 - DNA, 101 bp, Artificial Sequence
  ra74863s01, marker
ttctccttttgttctcgctacgcaaccagtaatttttttgtcttgagaatmtcacttttagcattttggtaggcactaaacatgaccagtgatgcataagg

SEQ ID NO: 253 - DNA, 101 bp, Artificial Sequence
  ra74864s01, marker
acttttctcaaaaagtaaatttgatgtttgtgttatgatttatatatgtamtgctatttgttttgatgatattttctctaagcatttatcactgagattag

SEQ ID NO: 254 - DNA, 101 bp, Artificial Sequence
  ra74865s01, marker
tgcattttctccaagatattcctttgctctccaaatctccacgagtgcagytcagcatcttgactccacatggtcttcaccattcaacatgtcatctgcgt

SEQ ID NO: 255 - DNA, 101 bp, Artificial Sequence
  ra74867s01, marker
tcatgaacatttagctgtttcagccatgactccgctgctcttccaagatamactaaccgctcttgatcaccagattctcgtttcccccacaaacctccttg

SEQ ID NO: 256 - DNA, 101 bp, Artificial Sequence
  ra74869s01, marker
aaaaaaacaaatctaacactataagtcccaatttttgataaaagaacaatyagtgacgaagaaatgatcaaagctagaagaagagagaagaatgattcaaa

SEQ ID NO: 257 - DNA, 101 bp, Artificial Sequence
  ra74870s01, marker
aaattccatattcactaggaaacttgtcccgtctcacaaatcttcttcttkctgagaatcacttgagaggtgaagttccgcctacaattggcaacctaaac

SEQ ID NO: 258 - DNA, 101 bp, Artificial Sequence
  ra74871s01, marker
attacgaaggtattcgaggttcgttatacatgggggcaatcaatcatacgkattcgatggatatgatgtataaaggtgtagacacagagtttccactgatc

SEQ ID NO: 259 - DNA, 101 bp, Artificial Sequence
  ra74915s01, marker
caaartacagacgtagagacagaatcagggtcaataaggaggagaggacakgaactcactctaatgaatactggagaaggctgttcamtgaagacatcttc

SEQ ID NO: 260 - DNA, 101 bp, Artificial Sequence
  ra74916s01, marker
ckcctcgtgtcgagcttcacacatctccgtcgtacggccattctcaggtakaaagcgttttctcgtttctcctctrtcgagkttgwgctcgatttgatatg

SEQ ID NO: 261 - DNA, 101 bp, Artificial Sequence
  ra74917s01, marker
cgtttgattccttgagaattttttttttttaaccttgagtttgtgtctaarttggattaatggtgtagaataagatttgaatacgagtatttttattccgt

SEQ ID NO: 262 - DNA, 101 bp, Artificial Sequence
  ra74919s01, marker
aaaactatgaagagcgtgtggcgtaagggagatgctgttgcagctgtggaraaagttgttaagcaagaacctaaaattgatagtaggggaccacctcagcc

SEQ ID NO: 263 - DNA, 101 bp, Artificial Sequence
  ra74921s01, marker
aataattaagaactgggtactggttctcattacctatacacacgttccttrcgacgattaaggtcgtgtgttacagttcagttcttaattycaaacatatt

SEQ ID NO: 264 - DNA, 101 bp, Artificial Sequence
  ra74922s01, marker
tttttaatttttaaagcttwtaaatttgggatgtaggtatttgtctctgcrgagcaattataaagacatgagtttaaaaaagtgttgtagactttaaaaaa

SEQ ID NO: 265 - DNA, 101 bp, Artificial Sequence
  ra74938s01, marker
atcctgagctcttgcacagataccggtgacattaggtatgtcaccacatcrttcctggagccctttagtatattcctggtctcatcatccttttggcatat

SEQ ID NO: 266 - DNA, 101 bp, Artificial Sequence
  ra74941s01, marker
ggagaggagagaggagagtcagtgttataaaacgacacgatatcctcacckagttacgcctcatttcctctcactccatctctctctctctctgtgttgtg

SEQ ID NO: 267 - DNA, 101 bp, Artificial Sequence
  ra74949s01, marker
aaatacacataacaaacagaatcttgcattgctacagatactagaaaaackagaaaccacttctttatatacaaatatgtacatgcagttgccttccccct

SEQ ID NO: 268 - DNA, 101 bp, Artificial Sequence
  ra74932s02, marker
ctctttgacaccgataggaatagtatcattcgctccaccgctgccttgaaytgtttcaatttctcaaactgctctgatcttcgttgccgcggaagagaacc

SEQ ID NO: 269 - DNA, 101 bp, Artificial Sequence
  ra74955s01, marker
acgcaaaagaacctgaaggtatgctttatcctcctcagttgacacaggtcwctctttatagagcttatatgttggtttaaatttgctatacactccataac

SEQ ID NO: 270 - DNA, 101 bp, Artificial Sequence
  ra74945s01, marker
gagagaacaaaagtcataatctggagctggacatctgggaatctaaatatmggaaagaatgttaagttttgatcacataaaacatgatatgatgaaaaaaa

SEQ ID NO: 271 - DNA, 101 bp, Artificial Sequence
  ra74946s01, marker
ataaacgtttatatcttgcgtagcatttcttaactcacacattgcttgtcrattatttggatcaggaatcaagttctcagttggcaatgggagcagctttt

SEQ ID NO: 272 - DNA, 101 bp, Artificial Sequence
  ra74948s01, marker
atgctgtgtccaggcgtagggttcgtcatcttgatgttcgtaatgagttgkataatgggatacttaagatgcctccgtctctctattcgtgtgagagattg

SEQ ID NO: 273 - DNA, 101 bp, Artificial Sequence
  ra74952s01, marker
cccccactgacgcctatactcggtccatctcttccctgagcggtgacagtytctgtgttcattacttcctcgccgtcatttatgctgctaatgcctgcttc

SEQ ID NO: 274 - DNA, 101 bp, Artificial Sequence
  ra74910s01, marker
ttaggccacgtaagctgcgagaaagctgtggtcacaactgccttcagtagrtttaccaatctgggtgtcaggactaacaagaagaagagaatcggtccggt

SEQ ID NO: 275 - DNA, 101 bp, Artificial Sequence
  ra01867s01, marker
caaaatcagamactgatggagaagaacataaagtagcaaaggagccagctkscaaagctgatggagtagagcgagagtctgtgaaagagccaratgaagaa

SEQ ID NO: 276 - DNA, 89 bp, Artificial Sequence
  ra01868s01, marker
ttaaagtctactacaaacaagtcaaatgcaaaatcagamactgatggagaagaacataaagtagcaaaggagccagctkscaaagctga

SEQ ID NO: 277 - DNA, 101 bp, Artificial Sequence
  ra13870s01, marker
  misc_feature (30)..(30): n is a, c, g, or t
  misc_feature (36)..(36): n is a, c, g, or t
  misc_feature (43)..(43): n is a, c, g, or t
tcawagaaacaaggctgagaatatcagttnaaaaangttacankttatgtrtgtccaaagaacaatatgcctcttagtaactcagactaaacaaagttaag

SEQ ID NO: 278 - DNA, 101 bp, Artificial Sequence
  ra17237s01, marker
ggtgttttatgtttttgkctagcttccctcgtagacaccttatagrcytgkgctacccggtttaggatcgctaatttctctgaaacgctttctttagtcac

SEQ ID NO: 279 - DNA, 101 bp, Artificial Sequence
  ra36486s01, marker
atcaatcggagatataaaaaatgataccaatagcataataacaaagatatktgatttaaaaagaaacttamaaaagtgatagrgtatccagatttcacatm

SEQ ID NO: 280 - DNA, 101 bp, Artificial Sequence
  ra36162s01, marker
tttgcaagtttttttctctcattgcgatcccctttcattcgtacttaccgyagaaataatgaaattaaaggatttrataactaactaatatyggtcamgta

SEQ ID NO: 281 - DNA, 101 bp, Artificial Sequence
  ra36410s01, marker
tccacacacacrtacyccactgatccttccaacrttcattaactttttctrattctcacattctgcagaaaataactttgttgcatcaccatgaagtcaaa

SEQ ID NO: 282 - DNA, 101 bp, Artificial Sequence
  ra36412s01, marker
tatgattggttwatgtttccmtttttcactccaatctrttgacatgataaygctcttactgaatagtttctcatggaacagttctgcatagctctagtgac

SEQ ID NO: 283 - DNA, 101 bp, Artificial Sequence
  ra36483s01, marker
catccatgatctttctcttctttgtaactttggcctmctctgtgctcactytcatgagtttcttctctgtttccacgcaaagaaccccatattactctgtt

SEQ ID NO: 284 - DNA, 101 bp, Artificial Sequence
  ra74872s01, marker
gttattacgttttcaaatatagcaaaaatatcacctaatgaggaataatayttacttggagtgaagtaatgatcttttccctttgatcaaagatattttgt

SEQ ID NO: 285 - DNA, 101 bp, Artificial Sequence; identical to SEQ ID NO: 274
  ra74910s01, marker

SEQ ID NO: 286 - DNA, 99 bp, Artificial Sequence
  ra74958s01, marker
ttgcttctttctcctttactgcaccttgtactctctctctctctctcaycattttcgaggtagtgagagagtgagatgcctgaaaccaaactcatttct

SEQ ID NO: 287 - DNA, 101 bp, Artificial Sequence
  ra74958s02, marker
gggattttgctgactcacttctcattgggaatattcttcatatgtttggcwtactgaaatttatgcaatcaactttgcattttaaattacaatcgtgtaat

SEQ ID NO: 288 - DNA, 99 bp, Artificial Sequence
  ra74958s03, marker
gggaaattcttctgacattcatcagagtgcaaacaacattttgtttggyaaactatagtctacagcttaatgatacagatcttccttggaaggaatata

SEQ ID NO: 289 - DNA, 101 bp, Artificial Sequence
  ra74958s04, marker
agtatcttactttatccggttcatcactaattgaaatgcattcattagaasaccgtgtaaaaaaagattcattcattataattaacgttttaacagtacca

SEQ ID NO: 290 - DNA, 99 bp, Artificial Sequence
  ra74958s05, marker
tagatcctctagtgacaacgttgaagccacctcgtcgaaytggagtatmgcagcttgctacaaaagaaacaacaatggtttaaaggcgcaattctcaag

SEQ ID NO: 291 - DNA, 101 bp, Artificial Sequence
  ra74958s06, marker
agtatcgcagcttgctacaaaagaaacaacaatggtttaaaggcgcaattmtcaaggtgactttatgcattaagttaaccaaagacgatccacttaccacg

SEQ ID NO: 292 - DNA, 101 bp, Artificial Sequence
  ra74958s07, marker
cttgctacaaaagaaacaacaatggtttaaaggcgcaattmtcaaggtgamtttatgcattaagttaaccaaagacgatccacttaccacgttcattatat

SEQ ID NO: 293 - DNA, 101 bp, Artificial Sequence
  ra74958s08, marker
acaatgtcaagatctccttcgaaggggcaccaactaacctaaagagagttsgtagtaacaaaaattcataagggattcacaaaaaaacaacgaatatctca